European Patent Specification EP 3 582 609 B1, published December 3, 2025. Title: Methods of targeted genetic alteration in plant cells. Applicant: Keygene N.V. The sequence listing filed with the application follows.

SEQUENCE LISTING (38 sequences)

SEQ ID NO: 1 - DNA, 5082 bp, Artificial Sequence
  DNA sequence encoding the rAPOBEC-Cas9-UGI fusion protein
atgggtagcagccatcatcatcaccatcatatgagcagcgaaacaggtccggttgcagttgatccgaccctgcgtcgtcgtattgaaccgcatgaatttgaagttttttttgatccgcgtgagctgcgtaaagaaacctgtctgctgtatgaaattaactggggtggtcgtcatagcatttggcgtcataccagccagaataccaataaacatgtggaagtgaacttcatcgagaaatttaccaccgaacgttatttttgtccgaatacccgttgtagcattacctggtttctgagctggtcaccgtgtggtgaatgtagccgtgcaattaccgaatttctgagccgttatccgcatgttaccctgtttatctatattgcccgtctgtatcatcatgcagatccgcgtaatcgtcagggtctgcgtgatctgattagcagcggtgttaccattcagattatgaccgaacaagaaagcggttattgctggcgtaattttgtgaattatagcccgagcaatgaagcacattggcctcgctatccgcatctgtgggttcgtctgtatgttctggaactgtattgtattattctgggtctgcctccgtgtctgaatattctgcgtcgtaaacagccgcagctgaccttttttaccattgcactgcagagctgtcattatcagcgtctgccaccgcatattctgtgggcaacaggtctgaaaagcggtagcgaaacaccgggtacaagcgaaagcgcaacaccggaaagcgacaaaaaatacagcattggtctggacattggtaccaacagcgtgggctgggccgtgatcaccgacgagtacaaggtgcccagcaagaagttcaaggtgctgggcaacaccgaccgccacagcatcaagaagaacctgatcggcgccctgctgttcgacagcggcgagaccgccgaggccacccgcctgaagcgcaccgcccgccgccgctacacccgccgcaagaaccgcatctgctacctgcaggagatcttcagcaacgagatggccaaggtggacgacagcttcttccaccgcctggaggagagcttcctggtggaggaggacaagaagcacgagcgccaccccatcttcggcaacatcgtggacgaggtggcctaccacgagaagtaccccaccatctaccacctgcgcaagaagctggtggacagcaccgacaaggccgacctgcgcctgatctacctggccctggcccacatgatcaagttccgcggccacttcctgatcgagggcgacctgaaccccgacaacagcgacgtggacaagctgttcatccagctggtgcagacctacaaccagctgttcgaggagaaccccatcaacgccagcggcgtggacgccaaggccatcctgagcgcccgcctgagcaagagccgccgcctggagaacctgatcgcccagctgcccggcgagaagaagaacggcctgttcggcaacctgatcgccctgagcctgggcctgacccccaacttcaagagcaacttcgacctggccgaggacgccaagctgcagctgagcaaggacacctacgacgacgacctggacaacctgctggcccagatcggcgaccagtacgccgacctgttcctggccgccaagaacctgagcgacgccatcctgctgagcgacatcctgcgcgtgaacaccgagatcaccaaggcccccctgagcgccagcatgatcaagcgctacgacgagcaccaccaggacctgaccctgctgaaggccctggtgcgccagcagctgcccgagaagtacaaggagatcttcttcgaccagagcaagaacggctacgccggctacatcgacggcggcgccagccaggaggagttctacaagttcatcaagcccatcctggagaagatggacggcaccgaggagctgctggtgaagctgaaccgcgaggacctgctgcgcaagcagcgcaccttcgacaacggcagcatcccccaccagatccacctgggcgagctgcacgccatcctgcgccgccaggaggacttctaccccttcctgaaggacaaccgcgagaagatcgagaagatcctgaccttccgcatcccctactacgtgggccccctggcccgcggcaacagccgcttcgcctggatgacccgcaagagcgaggagaccatcaccccctggaacttcgaggaggtggtggacaagggcgccagcgcccagagcttcatcgagcgcatgaccaacttcgacaagaacctgcccaacgagaaggtgctgcccaagcacagcctgctgtacgagtacttcaccgtgtacaacgagctgaccaaggtgaagtacgtgaccgagggcatgcgcaagcccgccttcctgagcggcgagcagaagaaggccatcgtggacctgctgttcaagaccaaccgcaaggtgaccgtgaagcagctgaaggaggactacttcaagaagatcgagtgcttcgacagcgtggagatcagcggcgtggaggaccgcttcaacgccagcctgggcacctaccacgacctgctgaagatcatcaaggacaaggacttcctggacaacgaggagaacgaggacatcctggaggacatcgtgctgaccctgaccctgttcgaggaccgcgagatgatcgaggagcgcctgaagacctacgcccacctgttcgacgacaaggtgatgaagcagctgaagcgccgccgctacaccggctggggccgcctgagccgcaagcttatcaacggcatccgcgacaagcagagcggcaagaccatcctggacttcctgaagagcgacggcttcgccaaccgcaacttcatgcagctgatccacgacgacagcctgaccttcaaggaggacatccagaaggcccaggtgagcggccagggcgacagcctgcacgagcacatcgccaacctggccggcagccccgccatcaagaagggcatcctgcagaccgtgaaggtggtggacgagctggtgaaggtgatgggccgccacaagcccgagaacatcgtgatcgagatggcccgcgagaaccagaccacccagaagggccagaagaacagccgcgagcgcatgaagcgcatcgaggagggcatcaaggagctgggcagccagatcctgaaggagcaccccgtggagaacacccagctgcagaacgagaagctgtacctgtactacctgcagaacggccgcgacatgtacgtggaccaggagctggacatcaaccgcctgagcgactacgacgtggaccacatcgtgccccagagcttcctgaaggacgacagcatcgacaacaaggtgctgacccgcagcgacaagaaccgcggcaagagcgacaacgtgcccagcgaggaggtggtgaagaagatgaagaactactggcgccagctgctgaacgccaagctgatcacccagcgcaagttcgacaacctgaccaaggccgagcgcggcggcctgagcgagctggacaaggccggcttcatcaagcgccagctggtggagacccgccagatcaccaagcacgtggcccagatcctggacagccgcatgaacaccaagtacgacgagaacgacaagctgatccgcgaggtgaaggtgatcaccctgaagagcaagctggtgagcgacttccgcaaggacttccagttctacaaggtgcgcgagatcaacaactaccaccacgcccacgacgcctacctgaacgccgtggtgggcaccgccctgatcaagaagtaccccaagctggagagcgagttcgtgtacggcgactacaaggtgtacgacgtgcgcaagatgatcgccaagagcgagcaggagatcggcaaggccaccgccaagtacttcttctacagcaacatcatgaacttcttcaagaccgagatcaccctggccaacggcgagatccgcaagcgccccctgatcgagaccaacggcgagaccggcgagatcgtgtgggacaagggccgcgacttcgccaccgtgcgcaaggtgctgagcatgccccaggtgaacatcgtgaagaagaccgaggtgcagaccggcggcttcagcaaggagagcatcctgcccaagcgcaacagcgacaagctgatcgcccgcaagaaggactgggaccccaagaagtacggcggcttcgacagccccaccgtggcctacagcgtgctggtggtggccaaggtggagaagggcaagagcaagaagctgaagagcgtgaaggagctgctgggcatcaccatcatggagcgcagcagcttcgagaagaaccccatcgacttcctggaggccaagggctacaaggaggtgaagaaggacctgatcatcaagctgcccaagtacagcctgttcgagctggagaacggccgcaagcgcatgctggccagcgccggcgagctgcagaagggcaacgagctggccctgcccagcaagtacgtgaacttcctgtacctggccagccactacgagaagctgaagggcagccccgaggacaacgagcagaagcagctgttcgtggagcagcacaagcactacctggacgagatcatcgagcagatcagcgagttcagcaagcgcgtgatcctggccgacgccaacctggacaaggtgctgagcgcctacaacaagcaccgcgacaagcccatccgcgagcaggccgagaacatcatccacctgttcaccctgaccaacctgggcgcccccgccgccttcaagtacttcgacaccaccatcgaccgcaagcgctacaccagcaccaaggaggtgctggacgccaccctgatccaccagagcatcaccggtctgtatgaaacccgtattgatctgagccagctgggtggtgatagcggtggtagcaccaatctgagcgatatcattgaaaaagaaaccggcaaacagctggtgattcaagaaagcattctgatgctgcctgaagaagtggaagaagttattggtaataaaccggaaagcgatattctggttcataccgcatatgatgaaagcaccgatgaaaatgttatgctgagcggtggttccccgaaaaaaaaacgtaaagtttaa

SEQ ID NO: 2 - protein, 1693 aa, Artificial Sequence
  rAPOBEC-Cas9-UGI fusion protein
MGSSHHHHHHMSSETGPVAVDPTLRRRIEPHEFEVFFDPRELRKETCLLYEINWGGRHSIWRHTSQNTNKHVEVNFIEKFTTERYFCPNTRCSITWFLSWSPCGECSRAITEFLSRYPHVTLFIYIARLYHHADPRNRQGLRDLISSGVTIQIMTEQESGYCWRNFVNYSPSNEAHWPRYPHLWVRLYVLELYCIILGLPPCLNILRRKQPQLTFFTIALQSCHYQRLPPHILWATGLKSGSETPGTSESATPESDKKYSIGLDIGTNSVGWAVITDEYKVPSKKFKVLGNTDRHSIKKNLIGALLFDSGETAEATRLKRTARRRYTRRKNRICYLQEIFSNEMAKVDDSFFHRLEESFLVEEDKKHERHPIFGNIVDEVAYHEKYPTIYHLRKKLVDSTDKADLRLIYLALAHMIKFRGHFLIEGDLNPDNSDVDKLFIQLVQTYNQLFEENPINASGVDAKAILSARLSKSRRLENLIAQLPGEKKNGLFGNLIALSLGLTPNFKSNFDLAEDAKLQLSKDTYDDDLDNLLAQIGDQYADLFLAAKNLSDAILLSDILRVNTEITKAPLSASMIKRYDEHHQDLTLLKALVRQQLPEKYKEIFFDQSKNGYAGYIDGGASQEEFYKFIKPILEKMDGTEELLVKLNREDLLRKQRTFDNGSIPHQIHLGELHAILRRQEDFYPFLKDNREKIEKILTFRIPYYVGPLARGNSRFAWMTRKSEETITPWNFEEVVDKGASAQSFIERMTNFDKNLPNEKVLPKHSLLYEYFTVYNELTKVKYVTEGMRKPAFLSGEQKKAIVDLLFKTNRKVTVKQLKEDYFKKIECFDSVEISGVEDRFNASLGTYHDLLKIIKDKDFLDNEENEDILEDIVLTLTLFEDREMIEERLKTYAHLFDDKVMKQLKRRRYTGWGRLSRKLINGIRDKQSGKTILDFLKSDGFANRNFMQLIHDDSLTFKEDIQKAQVSGQGDSLHEHIANLAGSPAIKKGILQTVKVVDELVKVMGRHKPENIVIEMARENQTTQKGQKNSRERMKRIEEGIKELGSQILKEHPVENTQLQNEKLYLYYLQNGRDMYVDQELDINRLSDYDVDHIVPQSFLKDDSIDNKVLTRSDKNRGKSDNVPSEEVVKKMKNYWRQLLNAKLITQRKFDNLTKAERGGLSELDKAGFIKRQLVETRQITKHVAQILDSRMNTKYDENDKLIREVKVITLKSKLVSDFRKDFQFYKVREINNYHHAHDAYLNAVVGTALIKKYPKLESEFVYGDYKVYDVRKMIAKSEQEIGKATAKYFFYSNIMNFFKTEITLANGEIRKRPLIETNGETGEIVWDKGRDFATVRKVLSMPQVNIVKKTEVQTGGFSKESILPKRNSDKLIARKKDWDPKKYGGFDSPTVAYSVLVVAKVEKGKSKKLKSVKELLGITIMERSSFEKNPIDFLEAKGYKEVKKDLIIKLPKYSLFELENGRKRMLASAGELQKGNELALPSKYVNFLYLASHYEKLKGSPEDNEQKQLFVEQHKHYLDEIIEQISEFSKRVILADANLDKVLSAYNKHRDKPIREQAENIIHLFTLTNLGAPAAFKYFDTTIDRKRYTSTKEVLDATLIHQSITGLYETRIDLSQLGGDSGGSTNLSDIIEKETGKQLVIQESILMLPEEVEEVIGNKPESDILVHTAYDESTDENVMLSGGSPKKKRKV

SEQ ID NO: 3 - DNA, 5328 bp, Artificial Sequence
  DNA sequence encoding the TadA-Cas9 D10A-NLS fusion protein
atgtccgaggtcgagttctctcatgagtactggatgaggcacgctctcactcttgctaaaagagcttgggacgagagagaggttccagttggagctgttttggtgcacaacaaccgtgtgattggcgaaggatggaacaggccaattggaaggcatgatccaactgctcacgctgagattatggcccttagacaaggtggactcgtgatgcagaactacaggcttatcgacgccactctctacgtgacacttgagccatgtgttatgtgcgctggtgccatgattcactccaggattggaagggttgtgttcggagctagagatgctaaaactggcgctgccggatctctcatggatgtgcttcatcatcctgggatgaaccacagggttgagatcactgagggaatccttgctgatgagtgcgctgctctcctgtctgattttttcaggatgaggcgtcaagagatcaaggcccagaagaaggctcagtcctctactgattctggcggatcttctggtgggtcatctggatctgaaacccctggaacttctgagtccgctactccagaatcatccggtggatctagtggtggttctagcgaggttgagttcagccacgaatactggatgcgtcacgcacttactttggctaagagggctcgtgatgagagggaagttcctgttggtgcagtgctcgtgcttaacaacagagtgatcggagaaggctggaatcgtgctatcggacttcatgatcctaccgcacatgcagagatcatggctttgaggcaaggtgggcttgtcatgcaaaattaccgtctgatcgacgctaccttgtacgtcacattcgagccttgcgtgatgtgtgctggggctatgatccattctaggatcggtagagtggtgttcggtgtgaggaatgctaagacaggtgctgctggctcacttatggatgtgttgcattaccccggcatgaaccaccgtgtggaaattacagagggcatcttggcagatgagtgtgccgctcttttgtgctacttcttcaggatgccacgtcaggtgttcaacgctcaaaagaaggcccaatccagcaccgattctggtggtagtagtggtggatcttccggatcagagactcctggtactagtgagtctgctacccctgaaagtagcggaggttcaagtggtgggtccgacaagaagtactctatcggattggctatcgggaccaactctgttggatgggctgtgatcactgacgagtacaaggtgccctccaagaagttcaaggttctcggaaacaccgacaggcactccatcaagaagaacctcatcggggctctgcttttcgattcaggtgaaactgctgaggccaccaggcttaagagaactgctagaagaaggtacacccgtaggaagaacaggatctgctacctccaagagatcttctccaacgagatggctaaggtggacgactcattcttccacaggctcgaagagtccttcttggtggaagaggataagaagcacgagaggcacccaatcttcgggaacattgtggatgaagtggcctaccacgagaagtacccaaccatctaccacctgaggaagaagctcgttgactccaccgataaggctgacctgaggcttatctaccttgctctcgctcacatgatcaagttccgtgggcacttccttatcgaaggggatctgaacccagacaactccgatgtggacaagctgttcattcagctcgtgcagacctacaaccagctgttcgaagagaacccaatcaacgcttctggtgtggacgctaaggctatcctttctgccaggctttccaagtccagaaggcttgagaacctgattgctcagcttcctggggagaagaagaacggacttttcgggaacctgatcgccctctctcttggacttactcccaacttcaagtccaacttcgacctcgctgaggatgccaagcttcagctctctaaggatacctacgatgacgacctcgacaacctccttgctcagattggagatcagtacgccgaccttttcctcgccgctaaaaacctctctgacgccatcctcctgtccgatattcttagggtgaacaccgagatcaccaaggcaccactttccgcctctatgatcaagcgttacgatgagcaccaccaggacctcactttgcttaaggctcttgttaggcagcagctcccagagaagtacaaagagattttcttcgaccagtccaagaacgggtacgccggttatattgatggtggggcttctcaagaagagttctacaagttcatcaagcccatcttggaaaagatggacgggaccgaagagttgctcgtgaagcttaaccgtgaggaccttcttaggaagcagcgaactttcgacaacggctctattcctcaccagatccaccttggagagctgcacgctattcttcgtaggcaagaggacttctacccattcctcaaggacaaccgtgagaagatcgagaagattctcaccttcaggatcccttactacgtgggaccacttgctaggggaaattctaggttcgcttggatgacccgtaagagcgaagagactatcactccatggaacttcgaagaggtggtggacaaaggtgctagcgctcagtctttcatcgagaggatgactaacttcgacaagaacctgccaaacgagaaggtgctcccaaagcactctctgctctacgagtacttcaccgtgtacaacgagctgaccaaggtcaagtatgtgaccgagggaatgcgtaagccagctttccttagtggtgagcagaaaaaggccatcgtggacctcttgttcaagaccaatagaaaggtgaccgtgaagcagctcaaagaggactacttcaaaaagatcgagtgcttcgactccgtcgagatctctggtgttgaggataggttcaacgcctccttgggaacttaccacgacctcctcaagatcatcaaggataaggatttcttggacaacgaggaaaacgaggacatcttggaggacatcgtgctcacccttaccttgttcgaggatcgagagatgatcgaggaacgactcaagacctacgctcacctgttcgatgacaaggtcatgaagcagttgaagaggcgtaggtacactggatggggacgtttgtcccgtaagctcattaacggaatcagggacaagcagtccggcaagactatcctcgacttcctcaagtctgatgggttcgccaaccgtaacttcatgcagctcatccacgacgacagcctgacctttaaagaggacatccaaaaggcccaggtgtccggtcaaggcgattctcttcatgagcacattgctaacctcgctgggtcaccagctatcaagaagggaattctccagactgtgaaggtcgtggacgagttggttaaggtgatgggtagacacaagcccgagaacatcgtgattgagatggctcgtgagaaccagactactcagaaggggcagaagaactccagggaacgtatgaagaggatcgaagaggggatcaaagagctggggtcccagattcttaaagagcacccagttgagaacacccagctccagaatgagaagctctacctctactacctgcagaacggcagggatatgtacgtggaccaagagctggatatcaacaggctctccgactacgatgttgaccacattgtgccccagtctttcttgaaggacgactccatcgacaacaaggtgctcaccaggtctgataagaaccgtgggaagtctgacaacgtgccatctgaagaggtcgtgaagaagatgaagaactactggcgtcagctcctcaacgccaagcttattactcagaggaagttcgacaacttgaccaaggctgagcgtggtggactttccgaacttgataaggccggattcatcaagaggcagctcgtggaaactaggcagatcactaagcacgtggcccagatcttggactctaggatgaacaccaagtacgacgagaacgacaagctcatccgtgaggtgaaggtcatcaccctcaagagcaagctggtgtccgatttcagaaaggacttccaattctacaaggtgagagagatcaacaactaccatcacgctcacgacgcttaccttaacgctgttgttggaaccgctctcatcaaaaagtaccccaagctcgagtccgagttcgtgtacggtgattacaaggtgtacgacgtgcgtaagatgatcgccaagtcagagcaagagatcggtaaggctaccgccaagtatttcttctactccaacatcatgaatttcttcaagactgagatcaccctcgccaacggggagattagaaagaggccacttatcgagactaacggcgagactggtgaaatcgtgtgggataagggaagagacttcgccactgtgcgtaaggtgttgtctatgccacaggtgaacatcgtcaagaaaaccgaggttcagaccggcgggttctccaaagaatctatccttccaaagaggaactccgacaagctgatcgctaggaagaaggattgggacccaaaaaagtacggtgggttcgattctccaaccgtggcttactctgttcttgttgtggccaaggttgagaaggggaagtctaagaaactcaagtccgtgaaagagctgctcgggatcactatcatggaaaggtccagcttcgagaagaatccaatcgatttcctcgaggccaagggctacaaagaggtgaagaaggaccttatcatcaagctccccaagtacagcctcttcgagttggagaacggacgtaagaggatgcttgcttctgctggggaacttcagaagggaaacgaactcgctctgccctctaagtacgtgaacttcctgtacctcgcttcccactacgagaagcttaagggatctccagaggataacgagcaaaagcagcttttcgtcgagcagcacaagcactacctcgacgagattatcgagcagatctccgagttctccaagcgtgtgattctcgctgatgccaacttggacaaggtgttgagcgcttacaacaagcaccgtgacaagccaattagagagcaggctgagaacatcatccacctgttcactctcaccaaccttggtgctccagctgcctttaagtacttcgataccaccatcgaccgtaagaggtacacctccaccaaagaggttttggacgctacccttatccaccagtccatcactggactttacgagactaggatcgacctctcacagctcggtggtgactctggtggatcaccaaagaagaagaggaaggtctaa

SEQ ID NO: 4 - protein, 1775 aa, Artificial Sequence
  TadA-Cas9 D10A-NLS fusion protein
MSEVEFSHEYWMRHALTLAKRAWDEREVPVGAVLVHNNRVIGEGWNRPIGRHDPTAHAEIMALRQGGLVMQNYRLIDATLYVTLEPCVMCAGAMIHSRIGRVVFGARDAKTGAAGSLMDVLHHPGMNHRVEITEGILADECAALLSDFFRMRRQEIKAQKKAQSSTDSGGSSGGSSGSETPGTSESATPESSGGSSGGSSEVEFSHEYWMRHALTLAKRARDEREVPVGAVLVLNNRVIGEGWNRAIGLHDPTAHAEIMALRQGGLVMQNYRLIDATLYVTFEPCVMCAGAMIHSRIGRVVFGVRNAKTGAAGSLMDVLHYPGMNHRVEITEGILADECAALLCYFFRMPRQVFNAQKKAQSSTDSGGSSGGSSGSETPGTSESATPESSGGSSGGSDKKYSIGLAIGTNSVGWAVITDEYKVPSKKFKVLGNTDRHSIKKNLIGALLFDSGETAEATRLKRTARRRYTRRKNRICYLQEIFSNEMAKVDDSFFHRLEESFLVEEDKKHERHPIFGNIVDEVAYHEKYPTIYHLRKKLVDSTDKADLRLIYLALAHMIKFRGHFLIEGDLNPDNSDVDKLFIQLVQTYNQLFEENPINASGVDAKAILSARLSKSRRLENLIAQLPGEKKNGLFGNLIALSLGLTPNFKSNFDLAEDAKLQLSKDTYDDDLDNLLAQIGDQYADLFLAAKNLSDAILLSDILRVNTEITKAPLSASMIKRYDEHHQDLTLLKALVRQQLPEKYKEIFFDQSKNGYAGYIDGGASQEEFYKFIKPILEKMDGTEELLVKLNREDLLRKQRTFDNGSIPHQIHLGELHAILRRQEDFYPFLKDNREKIEKILTFRIPYYVGPLARGNSRFAWMTRKSEETITPWNFEEVVDKGASAQSFIERMTNFDKNLPNEKVLPKHSLLYEYFTVYNELTKVKYVTEGMRKPAFLSGEQKKAIVDLLFKTNRKVTVKQLKEDYFKKIECFDSVEISGVEDRFNASLGTYHDLLKIIKDKDFLDNEENEDILEDIVLTLTLFEDREMIEERLKTYAHLFDDKVMKQLKRRRYTGWGRLSRKLINGIRDKQSGKTILDFLKSDGFANRNFMQLIHDDSLTFKEDIQKAQVSGQGDSLHEHIANLAGSPAIKKGILQTVKVVDELVKVMGRHKPENIVIEMARENQTTQKGQKNSRERMKRIEEGIKELGSQILKEHPVENTQLQNEKLYLYYLQNGRDMYVDQELDINRLSDYDVDHIVPQSFLKDDSIDNKVLTRSDKNRGKSDNVPSEEVVKKMKNYWRQLLNAKLITQRKFDNLTKAERGGLSELDKAGFIKRQLVETRQITKHVAQILDSRMNTKYDENDKLIREVKVITLKSKLVSDFRKDFQFYKVREINNYHHAHDAYLNAVVGTALIKKYPKLESEFVYGDYKVYDVRKMIAKSEQEIGKATAKYFFYSNIMNFFKTEITLANGEIRKRPLIETNGETGEIVWDKGRDFATVRKVLSMPQVNIVKKTEVQTGGFSKESILPKRNSDKLIARKKDWDPKKYGGFDSPTVAYSVLVVAKVEKGKSKKLKSVKELLGITIMERSSFEKNPIDFLEAKGYKEVKKDLIIKLPKYSLFELENGRKRMLASAGELQKGNELALPSKYVNFLYLASHYEKLKGSPEDNEQKQLFVEQHKHYLDEIIEQISEFSKRVILADANLDKVLSAYNKHRDKPIREQAENIIHLFTLTNLGAPAAFKYFDTTIDRKRYTSTKEVLDATLIHQSITGLYETRIDLSQLGGDSGGSPKKKRKV

SEQ ID NO: 5 - DNA, 183 bp, Artificial Sequence
  LIN5 sgRNA1
ggagtgatcaaaagtcccacatcgatcaggtgatatatagcagcttagtttatataatgatagagtcgacatagcgattgcctgacgatgaaattaagaagttttagagctagaaatagcaagttaaaataaggctagtccgttatcaacttgaaaaagtggcaccgagtcggtgcttttttt

SEQ ID NO: 6 - DNA, 183 bp, Artificial Sequence
  LIN5 sgRNA2
ggagtgatcaaaagtcccacatcgatcaggtgatatatagcagcttagtttatataatgatagagtcgacatagcgattgttcatcgtcaggtaatacatgttttagagctagaaatagcaagttaaaataaggctagtccgttatcaacttgaaaaagtggcaccgagtcggtgcttttttt

SEQ ID NO: 7 - DNA, 183 bp, Artificial Sequence
  ALS2 sgRNA1
ggagtgatcaaaagtcccacatcgatcaggtgatatatagcagcttagtttatataatgatagagtcgacatagcgattgcaagtgccgaggaggatgatgttttagagctagaaatagcaagttaaaataaggctagtccgttatcaacttgaaaaagtggcaccgagtcggtgcttttttt

SEQ ID NO: 8 - DNA, 183 bp, Artificial Sequence
  ALS2 sgRNA2
ggagtgatcaaaagtcccacatcgatcaggtgatatatagcagcttagtttatataatgatagagtcgacatagcgattgcatcctcctcggcacttgacgttttagagctagaaatagcaagttaaaataaggctagtccgttatcaacttgaaaaagtggcaccgagtcggtgcttttttt

SEQ ID NO: 9 - DNA, 183 bp, Artificial Sequence
  ALS2 sgRNA3
ggagtgatcaaaagtcccacatcgatcaggtgatatatagcagcttagtttatataatgatagagtcgacatagcgattgttaccggtcaagtgccgagggttttagagctagaaatagcaagttaaaataaggctagtccgttatcaacttgaaaaagtggcaccgagtcggtgcttttttt

SEQ ID NO: 10 - DNA, 183 bp, Artificial Sequence
  ALS2 S640 sgRNA1
ggagtgatcaaaagtcccacatcgatcaggtgatatatagcagcttagtttatataatgatagagtcgacatagcgattggcaccgccactgggaatcatgttttagagctagaaatagcaagttaaaataaggctagtccgttatcaacttgaaaaagtggcaccgagtcggtgcttttttt

SEQ ID NO: 11 - DNA, 183 bp, Artificial Sequence
  ALS2 S640 sgRNA2
ggagtgatcaaaagtcccacatcgatcaggtgatatatagcagcttagtttatataatgatagagtcgacatagcgattgtctttgaaagcaccgccactgttttagagctagaaatagcaagttaaaataaggctagtccgttatcaacttgaaaaagtggcaccgagtcggtgcttttttt

SEQ ID NO: 12 - DNA, 183 bp, Artificial Sequence
  ALS2 S640 sgRNA3
ggagtgatcaaaagtcccacatcgatcaggtgatatatagcagcttagtttatataatgatagagtcgacatagcgattgctaccgatgattcccagtgggttttagagctagaaatagcaagttaaaataaggctagtccgttatcaacttgaaaaagtggcaccgagtcggtgcttttttt

SEQ ID NO: 13 - DNA, 23 bp, Artificial Sequence
  LIN5 target site
cctgacgatgaaattaagaaagg

SEQ ID NO: 14 - DNA, 23 bp, Artificial Sequence
  LIN5 target site
cctgacgatgaaattaagaaagg

SEQ ID NO: 15 - DNA, 23 bp, Artificial Sequence
  LIN5 target site
ccgatgtattacctgacgatgaa

SEQ ID NO: 16 - DNA, 23 bp, Artificial Sequence
  LIN5 target site
cctgacgatgaaattaagaaagg

SEQ ID NO: 17 - DNA, 23 bp, Artificial Sequence
  LIN5 target site
cctgacgatgaaattaagaaagg

SEQ ID NO: 18 - DNA, 20 bp, Artificial Sequence
  WT target sequence
atgtattacctgacgatgaa

SEQ ID NO: 19 - DNA, 20 bp, Artificial Sequence
  line 1 target sequence
atgtattayctgaygatgaa

SEQ ID NO: 20 - DNA, 20 bp, Artificial Sequence
  line 2 target sequence
atgtattacytgaygatgaa

SEQ ID NO: 21 - DNA, 20 bp, Artificial Sequence
  line 3 target sequence
atgtattayytgaygatgaa

SEQ ID NO: 22 - DNA, 20 bp, Artificial Sequence
  line 4 target sequence
atgtattacctgacratraa

SEQ ID NO: 23 - DNA, 20 bp, Artificial Sequence
  line 5 target sequence
atgtattacctracratraa

SEQ ID NO: 24 - DNA, 20 bp, Artificial Sequence
  line 6 target sequence
atgtattacctaacaataaa

SEQ ID NO: 25 - DNA, 39 bp, Artificial Sequence
  target site
tgctattaccggtcaagtgccgaggaggatgattggtac

SEQ ID NO: 26 - DNA, 39 bp, Artificial Sequence
  target site
acgataatggccagttcacggctcctcctactaaccatg

SEQ ID NO: 27 - DNA, 39 bp, Artificial Sequence
  target site
tgttctaccgatgattcccagtggcggtgctttcaaaga

SEQ ID NO: 28 - DNA, 39 bp, Artificial Sequence
  target site
acaagatggctactaagggtcaccgccacgaaagtttct

SEQ ID NO: 29 - DNA, 39 bp, Artificial Sequence; identical to SEQ ID NO: 25
  P184 ref

SEQ ID NO: 30 - DNA, 39 bp, Artificial Sequence; identical to SEQ ID NO: 27
  S640 ref

SEQ ID NO: 31 - DNA, 39 bp, Artificial Sequence; identical to SEQ ID NO: 27
  S640 ref

SEQ ID NO: 32 - protein, 11 aa, Artificial Sequence
  linker
SPKKKRKVEAS

SEQ ID NO: 33 - protein, 16 aa, Artificial Sequence
  linker
SGSETPGTSESATPES

SEQ ID NO: 34 - protein, 17 aa, Artificial Sequence
  linker
KSGSETPGTSESATPES

SEQ ID NO: 35 - DNA, 21 bp, Artificial Sequence
  forward primer
cactattggcatgtatcacac

SEQ ID NO: 36 - DNA, 22 bp, Artificial Sequence
  reversed primer
gtgatgctgagatccctttaac

SEQ ID NO: 37 - protein, 6 aa, Artificial Sequence
  His-tag
HHHHHH

SEQ ID NO: 38 - protein, 5 aa, Artificial Sequence
  linker
EAAAK